European Patent Specification EP 4 422 479 B1, published September 16, 2026. Title: CONTINUOUS CORTISOL MONITORING SYSTEM WITH MICRONEEDLE ARRAY. Applicant: Biolinq Incorparated. Application US. The sequence listing filed with the application follows.

SEQUENCE LISTING (1 sequence)

SEQ ID NO: 1 - DNA, 42 bp, synthetic construct
  source 1..42: mol_type = other DNA
ggacgacgccagaagtttacgaggatatggtaacatagtcgt